European Patent Application EP 4 685 154 A1, published January 28, 2026. Title: Polypeptide derived from tridegin. Applicant: Rheinische Friedrich-Wilhelms-Universität Bonn. Application EP. The sequence listing filed with the application follows.

SEQUENCE LISTING (11 sequences)

SEQ ID NO: 1 - protein, 66 aa, synthetic construct
  MOD_RES 1: note = Lys, D-Lys, Arg, D-Arg, Orn or citrulline
  MOD_RES 6: note = Lys, D-Lys, Arg, D-Arg, Orn or citrulline
  MOD_RES 16: note = Lys, D-Lys, Arg, D-Arg, Orn or citrulline
  MOD_RES 38: note = Lys, D-Lys, Arg, D-Arg, Orn or citrulline
  MOD_RES 40: note = Lys, D-Lys, Arg, D-Arg, Orn or citrulline
  MOD_RES 45: note = Lys, D-Lys, Arg, D-Arg, Orn or citrulline
  MOD_RES 53: note = Lys, D-Lys, Arg, D-Arg, Orn or citrulline
  MOD_RES 63: note = Lys, D-Lys, Arg, D-Arg, Orn or citrulline
  MOD_RES 65: note = Lys, D-Lys, Arg, D-Arg, Orn or citrulline
  MOD_RES 5: note = Ser, Ala, Cys, S-methylcysteine, or amino acid moiety capable of forming a lactam bond
  MOD_RES 17: note = Ser, Ala, Cys, S-methylcysteine, or amino acid moiety capable of forming a lactam bond
  MOD_RES 31: note = Ser, Ala, Cys, S-methylcysteine, or amino acid moiety capable of forming a lactam bond
  MOD_RES 37: note = Ser, Ala, Cys, S-methylcysteine, or amino acid moiety capable of forming a lactam bond
  MOD_RES 19: note = Ala or S-methylcysteine
  MOD_RES 25: note = Ala or S-methylcysteine
XLLPXXEWHQGIPNPXXWXGADLEXAQDQYXAFIPQXXPXSELIXPMDDIYQXPVEFPNLPLXPXE

SEQ ID NO: 2 - protein, 66 aa, synthetic construct
  SITE 6: note = D-lysine
  SITE 12: note = D-isoleucine
  SITE 23: note = D-leucine
  SITE 34: note = D-isoleucine
  DISULFID 5..37: note = potential intrachain disulfide bond
  DISULFID 17..31: note = potential intrachain disulfide bond
KLLPCKEWHQGIPNPRCWSGADLESAQDQYCAFIPQCRPRSELIKPMDDIYQRPVEFPNLPLKPRE

SEQ ID NO: 3 - protein, 66 aa, synthetic construct
  MOD_RES 1: note = Orn
  MOD_RES 6: note = Orn
  MOD_RES 45: note = Orn
  MOD_RES 63: note = Orn
  MOD_RES 16: note = citrulline
  MOD_RES 38: note = citrulline
  MOD_RES 40: note = citrulline
  MOD_RES 53: note = citrulline
  MOD_RES 65: note = citrulline
XLLPSXEWHQGIPNPXSWSGADLESAQDQYSAFIPQSXPXSELIXPMDDIYQXPVEFPNLPLXPXE

SEQ ID NO: 4 - protein, 66 aa, synthetic construct
KLLPAKEWHQGIPNPRAWAGADLEAAQDQYAAFIPQARPRSELIKPMDDIYQRPVEFPNLPLKPRE

SEQ ID NO: 5 - protein, 66 aa, synthetic construct
  MOD_RES 1: note = Orn
  MOD_RES 6: note = Orn
  MOD_RES 45: note = Orn
  MOD_RES 63: note = Orn
  MOD_RES 16: note = citrulline
  MOD_RES 38: note = citrulline
  MOD_RES 40: note = citrulline
  MOD_RES 53: note = citrulline
  MOD_RES 65: note = citrulline
XLLPAXEWHQGIPNPXAWAGADLEAAQDQYAAFIPQAXPXSELIXPMDDIYQXPVEFPNLPLXPXE

SEQ ID NO: 6 - protein, 66 aa, synthetic construct; identical to SEQ ID NO: 2
  DISULFID 5..37: note = potential intrachain disulfide bond
  DISULFID 17..31: note = potential intrachain disulfide bond

SEQ ID NO: 7 - protein, 66 aa, synthetic construct
KLLPSKEWHQGIPNPRSWSGADLESAQDQYSAFIPQSRPRSELIKPMDDIYQRPVEFPNLPLKPRE

SEQ ID NO: 8 - protein, 66 aa, synthetic construct
KLLPSKEWHQGIPNPRSWAGADLEAAQDQYSAFIPQSRPRSELIKPMDDIYQRPVEFPNLPLKPRE

SEQ ID NO: 9 - protein, 66 aa, synthetic construct; identical to SEQ ID NO: 8
  SITE 1: note = D-lysine

SEQ ID NO: 10 - protein, 66 aa, synthetic construct; identical to SEQ ID NO: 8
  SITE 23: note = D-leucine

SEQ ID NO: 11 - protein, 66 aa, synthetic construct
  MOD_RES 19: note = S-methylcysteine
  MOD_RES 25: note = S-methylcysteine
KLLPSKEWHQGIPNPRSWXGADLEXAQDQYSAFIPQSRPRSELIKPMDDIYQRPVEFPNLPLKPRE